European Patent Application EP 4 674 380 A1, published January 7, 2026. Title: Support element for an artificial cornea. Applicant: Universitat Internacional de Catalunya. Application EP. The sequence listing filed with the application follows.

SEQUENCE LISTING (4 sequences)

SEQ ID NO: 1 - protein, 12 aa, synthetic construct
KRIWFIPRSSWY

SEQ ID NO: 2 - protein, 15 aa, synthetic construct
KRIWFIPRSSWYERA

SEQ ID NO: 3 - protein, 14 aa, synthetic construct
  SITE 13: note = (Acp)m wherein m is 1, 2 or 3
  SITE 14: note = (L-3,4-dihyroxylphenylalanine)n wherein n is 1, 2 or 3
  SITE 1: note = N-terminal end corresponds to -NHR2, wherein R2 is a radical selected from the group consisting of -H, -C(O)R5, wherein R5 is a radical independently selected from the group consisting of: -H and (C1-C10)alkyl.
  SITE 14: note = C-terminal end corresponds to to -C(O)R1, wherein R1 is a radical selected from the group consisting of -OH and -NR3R4, wherein R3, R4 are radicals independently selected from the group consisting of: -H and (C1-C10)alkyl.
KRIWFIPRSSWYXX

SEQ ID NO: 4 - protein, 17 aa, synthetic construct
  SITE 1: note = acetyl
  SITE 14: note = Acp
  SITE 15: note = Acp
  SITE 16: note = L-3,4-dihydroxyphenylalanine
  SITE 17: note = L-3,4-dihydroxyphenylalanine
KRIWIFIPRSSWYXXXX